European Patent Application EP 4 458 855 A1, published November 6, 2024. Title: DEVELOPMENT OF NOVEL PDL1 SINGLE-DOMAIN ANTIBODY. Applicant: PERSONGEN BIOTHERAPEUTICS (SUZHOU) CO., LTD. The sequence listing filed with the application follows.

SEQUENCE LISTING (37 sequences)

SEQ ID NO: 1 - protein, 124 aa, synthetic construct
  source 1..124: note = Nanoantibody 17-A06
MAQVKLEESGGGLVQAGGSLRLSCVASGRSFITYAVGWFRQAPGKEREFVASINWSGAMTYYTDSVNGRFAISRDNAKNTVYLQMNNLKLEDTAVYYCASTISAVTPTNGYQNWGQGTQVTVSS

SEQ ID NO: 2 - protein, 122 aa, synthetic construct
  source 1..122: note = Nanoantibody 17-C12
MAQVKLEESGGGLVQPGGSLTLSCAASGRTFGFYGWFRQAPGKEREFVAGITWGGSVTSYADSVKGRFTISRDNAKNTVYLQMNSLKPENTAVYYCARSPRVTTTPREFDVWGQGTQVTVSS

SEQ ID NO: 3 - protein, 122 aa, synthetic construct
  source 1..122: note = Nanoantibody 17-A01
MAAVQLVDSGGGLVQPGGSLRLSCAASGRTFGFYGWFRQAPGKEREFVAAITWGGSAISYEDSAKGRFTISRDNAKNTVYLQMNSLKPEDTAVYYCARSTRVTTNPREYDYWGQGTQVTVSS

SEQ ID NO: 4 - protein, 122 aa, synthetic construct
  source 1..122: note = Nanoantibody 17-G06
MAAVQLVESGGGLVQPGGSLRLSCAASGRTFGFYGWFRQAPGKEREFVAAITWGGSAISYDDSAKGRFTISRDNAKNTVYLQMNSLKPEDTAVYYCARSMRVTTNPREYDYWGQGTQVTVSS

SEQ ID NO: 5 - protein, 124 aa, synthetic construct
  source 1..124: note = Nanoantibody 23-G3
MAAVQLVESGGGLVQAGGSLRLSCVASGRSFITYAVGWFRQAPGKEREFVASVNWSGAMTYYADAVNGRFTISRDNAKNTVYLQMNNLKLEDTAVYYCAATISAVTPTNGYQNWGQGTQVTVSS

SEQ ID NO: 6 - protein, 114 aa, synthetic construct
  source 1..114: note = Nanoantibody 29-H9
RLQLVESGGGLVQAGGSLRLSCAASGFTFSTYAMSWYRGVPEKERELVAFISSDGGGTTYRDSVKGRFTISRDNGKNTVYLQMNSLKPEDTGVYYCARGLAQIWGQGTQVTVSS

SEQ ID NO: 7 - protein, 8 aa, synthetic construct
  source 1..8: note = CDR1 of nano antibody 17-A06, 23-G3
GRSFITYA

SEQ ID NO: 8 - protein, 8 aa, synthetic construct
  source 1..8: note = CDR2 of nano antibody 17-A06
INWSGAMT

SEQ ID NO: 9 - protein, 15 aa, synthetic construct
  source 1..15: note = CDR3 of nano antibody 17-A06
ASTISAVTPTNGYQN

SEQ ID NO: 10 - protein, 6 aa, synthetic construct
  source 1..6: note = CDR1 of nano antibody 17-C12, 17-A01, 17-G06
GRTFGF

SEQ ID NO: 11 - protein, 8 aa, synthetic construct
  source 1..8: note = CDR2 of nano antibody 17-C12
ITWGGSVT

SEQ ID NO: 12 - protein, 15 aa, synthetic construct
  source 1..15: note = CDR3 of nano antibody 17-C12
ARSPRVTTTPREFDV

SEQ ID NO: 13 - protein, 8 aa, synthetic construct
  source 1..8: note = CDR2 of nano antibody 17-A01, 17-G06
ITWGGSAI

SEQ ID NO: 14 - protein, 15 aa, synthetic construct
  source 1..15: note = CDR3 of nano antibody 17-A01
ARSTRVTTNPREYDY

SEQ ID NO: 15 - protein, 15 aa, synthetic construct
  source 1..15: note = CDR3 of nano antibody 17-G06
ARSMRVTTNPREYDY

SEQ ID NO: 16 - protein, 8 aa, synthetic construct
  source 1..8: note = CDR2 of nano antibody 23-G3
VNWSGAMT

SEQ ID NO: 17 - protein, 15 aa, synthetic construct
  source 1..15: note = CDR3 of nano antibody 23-G3
AATISAVTPTNGYQN

SEQ ID NO: 18 - protein, 8 aa, synthetic construct
  source 1..8: note = CDR1 of nano antibody 29-H9
GFTFSTYA

SEQ ID NO: 19 - protein, 8 aa, synthetic construct
  source 1..8: note = CDR2 of nano antibody 29-H9
ISSDGGGT

SEQ ID NO: 20 - protein, 7 aa, synthetic construct
  source 1..7: note = CDR3 of nano antibody 29-H9
ARGLAQI

SEQ ID NO: 21 - protein, 27 aa, synthetic construct
  source 1..27: note = FR1 of nano antibody 17-A06
MAQVKLEESGGGLVQAGGSLRLSCVAS

SEQ ID NO: 22 - protein, 17 aa, synthetic construct
  source 1..17: note = FR2 of nano antibody 17-A06, 23-G3
VGWFRQAPGKEREFVAS

SEQ ID NO: 23 - protein, 38 aa, synthetic construct
  source 1..38: note = FR3 of nano antibody 17-A06
YYTDSVNGRFAISRDNAKNTVYLQMNNLKLEDTAVYYC

SEQ ID NO: 24 - protein, 11 aa, synthetic construct
  source 1..11: note = FR4 of nano antibodies 17-A06, 17-C12, 17-A01, 17-G06, 23-G3, 29-H9
WGQGTQVTVSS

SEQ ID NO: 25 - protein, 27 aa, synthetic construct
  source 1..27: note = FR1 of nano antibody 17-C12
MAQVKLEESGGGLVQPGGSLTLSCAAS

SEQ ID NO: 26 - protein, 17 aa, synthetic construct
  source 1..17: note = FR2 of nano antibody 17-C12
YGWFRQAPGKEREFVAG

SEQ ID NO: 27 - protein, 38 aa, synthetic construct
  source 1..38: note = FR3 of nano antibody 17-C12
SYADSVKGRFTISRDNAKNTVYLQMNSLKPENTAVYYC

SEQ ID NO: 28 - protein, 27 aa, synthetic construct
  source 1..27: note = FR1 of nano antibody 17-A01
MAAVQLVDSGGGLVQPGGSLRLSCAAS

SEQ ID NO: 29 - protein, 17 aa, synthetic construct
  source 1..17: note = FR2 of nano antibody 17-A01, 17-G06
YGWFRQAPGKEREFVAA

SEQ ID NO: 30 - protein, 38 aa, synthetic construct
  source 1..38: note = FR3 of nano antibody 17-A01
SYEDSAKGRFTISRDNAKNTVYLQMNSLKPEDTAVYYC

SEQ ID NO: 31 - protein, 27 aa, synthetic construct
  source 1..27: note = FR1 of nano antibody 17-G06
MAAVQLVESGGGLVQPGGSLRLSCAAS

SEQ ID NO: 32 - protein, 38 aa, synthetic construct
  source 1..38: note = FR3 of nano antibody 17-G06
SYDDSAKGRFTISRDNAKNTVYLQMNSLKPEDTAVYYC

SEQ ID NO: 33 - protein, 27 aa, synthetic construct
  source 1..27: note = FR1 of nano antibody 23-G3
MAAVQLVESGGGLVQAGGSLRLSCVAS

SEQ ID NO: 34 - protein, 38 aa, synthetic construct
  source 1..38: note = FR3 of nano antibody 23-G3
YYADAVNGRFTISRDNAKNTVYLQMNNLKLEDTAVYYC

SEQ ID NO: 35 - protein, 25 aa, synthetic construct
  source 1..25: note = FR1 of nano antibody 29-H9
RLQLVESGGGLVQAGGSLRLSCAAS

SEQ ID NO: 36 - protein, 17 aa, synthetic construct
  source 1..17: note = FR2 of nano antibody 29-H9
MSWYRGVPEKERELVAF

SEQ ID NO: 37 - protein, 38 aa, synthetic construct
  source 1..38: note = FR3 of nano antibody 29-H9
TYRDSVKGRFTISRDNGKNTVYLQMNSLKPEDTGVYYC